European Patent Application EP 4 529 958 A2, published April 2, 2025. Title: CONTROLLABLE TRANSCRIPTION. Applicant: Cambridge Enterprise Limited. Application EP. The sequence listing filed with the application follows.

SEQUENCE LISTING (88 sequences)

SEQ ID NO: 1 - DNA, 19 bp, synthetic construct
  misc_feature 1..19: note = TetO2 19 nucleotide sequence
  source 1..19: mol_type = other DNA
tccctatcagtgatagaga

SEQ ID NO: 2 - DNA, 1797 bp, Homo sapiens
  source 1..1797: mol_type = genomic DNA
gctcgaaaccggacggagccattgctctcgcagagggaggagcgcttccggctagcctcttgtcgccgattggccgtttctcctcccgccgtgtgtgaaaacacaaatggcgtattctggttggagtaaagctcctgtcagttacgccgtcgggagtacgcagccgcttagcgactctcgcgttgccccctgggtggggcgggtaggtaggtggggtgtagagatgctgggtgtgcgggcgcggccggcctcctgcggcgggaggggagggtcagtgaaatcggctctggcgcgggcgtcctcccaccctccccttccttcgggggagtcggtttacccgccgcctgcttgtcttcgacacctgattggctgtcgaagctgtgggaccgggcccttgctactggctcgagtctcacatgagcgaaaccactgcgcggggcgcgggggtggcggggaggcgggcgttggtacggtcctccccgaggccgagcgccgcagtgtctggccccgcgcccctgcgcaacgtggcaggaagcgcgcgctggaggcgggggcgggctgccggccgagacttctggatggcggcggccgcggctccgccccgggttcccaccgcctgaagggcgagacaagcccgacctgctacaggcactcgtgggggtgggggaggagcgggggtcggtccggctggtttgtgggtgggaggcgcttgttctccaaaaaccggcgcgagctgcaatcctgagggagctgcggtggaggaggtggagagaaggccgcacccttctgggcagggggaggggagtgccgcaatacctttatgggagttctctgctgcctcccgtcttgtaaggaccgccctgggcctggaagaagccctccctcctttcctcctcgcgtgatctcgtcatcgcctccatgtcgagtcgcttctcgattatgggcgggattcttttgcctaggcttaaggggctaacttggtccctgggcgttgccctgcaggggagtgagcagctgtaagatttgaggggcgactccgattagtttatcttcccacggactagagttggtgtcgaggttattgtaataagggtggggtagggaaatggagcttagtcattcacctggggctgattttatgcaacgagactgcggattatcactacttatcatttttggagcatttttctagagacagacataaagcatgatcacctgagttttataccatttgagacccttgctgcaccaccaaagtgtagcatcaggttaaatcttaatagaaaaattttagcttttgcttgagaaaccagtgcttccctccctcaccctctctccccaggctctctacccctttgcatccctaccaggcatcttagcaactctcactcatacttgatcccattttccatttgttgtacttgctcctctagtattcagacatagcactagctttctccctctcttgatcttgggtagcctggtgtctcgcgaaaccagacagattggttccaccacaaattaaggcttgagctggggcttgactcttacccagcagtgcttttattcctccctagttcacgttcttaaatgtttatcttgattttcattttatcctttttccttagctgggattctgtccctgaccgtcttcacagtccaggtgatcttgactactgctttacagagaattggatctgaggttaggcaacatctccctttttcttcctctaaatacctctcatttctgttcttaccagttagtaactgatctcagatgcctgtgtgatagcttcc

SEQ ID NO: 3 - DNA, 651 bp, synthetic construct
  misc_feature 1..651: note = STDtetR-nls
  source 1..651: mol_type = other DNA
atgccaaaaaagaagaggaaggtatctagattagataaaagtaaagtgattaacagcgcattagagctgcttaatgaggtcggaatcgaaggtttaacaacccgtaaactcgcccagaagctaggtgtagagcagcctacattgtattggcatgtaaaaaataagcgggctttgctcgacgccttagccattgagatgttagataggcaccatactcacttttgccctttagaaggggaaagctggcaagattttttacgtaataacgctaaaagttttagatgtgctttactaagtcatcgcgatggagcaaaagtacatttaggtacacggcctacagaaaaacagtatgaaactctcgaaaatcaattagcctttttatgccaacaaggtttttcactagagaatgcattatatgcactcagcgctgtggggcattttactttaggttgcgtattggaagatcaagagcatcaagtcgctaaagaagaaagggaaacacctactactgatagtatgccgccattattacgacaagctatcgaattatttgatcaccaaggtgcagagccagccttcttattcggccttgaattgatcatatgcggattagaaaaacaacttaaatgtgaaagtgggtctccgcggtaa

SEQ ID NO: 4 - protein, 216 aa, synthetic construct [sequence omitted]

SEQ ID NO: 5 - DNA, 651 bp, synthetic construct
  misc_feature 1..651: note = OPTtetR
  source 1..651: mol_type = other DNA
atgcccaagaaaaagcggaaggtgtcccggctggacaagagcaaagtgatcaacagcgccctggaactgctgaacgaagtgggcatcgagggcctgaccacccggaagctggcccagaaactgggcgtggaacagcccaccctgtactggcacgtgaagaacaagcgggccctgctggacgccctggccatcgagatgctggaccggcaccacacacacttttgccccctggaaggcgaaagctggcaggacttcctgcggaacaacgccaagagcttcagatgcgccctgctgagccaccgggacggcgccaaagtgcacctgggcaccagacccaccgagaagcagtacgagacactggaaaaccagctggccttcctgtgccagcagggcttcagcctggaaaacgccctgtacgccctgagcgccgtgggccactttaccctgggctgcgtgctggaagatcaggaacaccaggtcgccaaagaggaaagagagacacccaccaccgacagcatgccccccctgctgagacaggccatcgagctgttcgatcatcaaggcgccgagcccgccttcctgttcggcctggaactgatcatctgcggcctcgagaagcagctgaagtgcgagagcggctcccccagatga

SEQ ID NO: 6 - protein, 216 aa, synthetic construct [sequence omitted]

SEQ ID NO: 7 - DNA, 20 bp, synthetic construct
  misc_feature 1..20: note = hROSA26 Locus PCR
  source 1..20: mol_type = other DNA
gagaagaggctgtgcttcgg

SEQ ID NO: 8 - DNA, 22 bp, synthetic construct
  misc_feature 1..22: note = hROSA26 Locus PCR
  source 1..22: mol_type = other DNA
acagtacaagccagtaatggag

SEQ ID NO: 9 - DNA, 20 bp, synthetic construct
  misc_feature 1..20: note = hROSA26 5'-INT PCR
  source 1..20: mol_type = other DNA
gagaagaggctgtgcttcgg

SEQ ID NO: 10 - DNA, 21 bp, synthetic construct
  misc_feature 1..21: note = hROSA26 5'-INT PCR
  source 1..21: mol_type = other DNA
aagaccgcgaagagtttgtcc

SEQ ID NO: 11 - DNA, 21 bp, synthetic construct
  misc_feature 1..21: note = hROSA26 3'-INT PCR
  source 1..21: mol_type = other DNA
gaaactcgctcaaaagctggg

SEQ ID NO: 12 - DNA, 22 bp, synthetic construct
  misc_feature 1..22: note = hROSA26 3'-INT PCR
  source 1..22: mol_type = other DNA
acagtacaagccagtaatggag

SEQ ID NO: 13 - DNA, 21 bp, synthetic construct
  misc_feature 1..21: note = hROSA26 3'-BB PCR
  source 1..21: mol_type = other DNA
gaaactcgctcaaaagctggg

SEQ ID NO: 14 - DNA, 20 bp, synthetic construct
  misc_feature 1..20: note = hROSA26 3'-BB PCR
  source 1..20: mol_type = other DNA
tgaccatgattacgccaagc

SEQ ID NO: 15 - DNA, 25 bp, synthetic construct
  misc_feature 1..25: note = AAVS1 Locus PCR
  source 1..25: mol_type = other DNA
ctgtttccccttcccaggcaggtcc

SEQ ID NO: 16 - DNA, 25 bp, synthetic construct
  misc_feature 1..25: note = AAVS1 Locus PCR
  source 1..25: mol_type = other DNA
tgcaggggaacggggctcagtctga

SEQ ID NO: 17 - DNA, 25 bp, synthetic construct
  misc_feature 1..25: note = AAVS1 5'-INT PCR
  source 1..25: mol_type = other DNA
ctgtttccccttcccaggcaggtcc

SEQ ID NO: 18 - DNA, 25 bp, synthetic construct
  misc_feature 1..25: note = AAVS1 5'-INT PCR
  source 1..25: mol_type = other DNA
tcgtcgcgggtggcgaggcgcaccg

SEQ ID NO: 19 - DNA, 25 bp, synthetic construct
  misc_feature 1..25: note = AAVS1 3'-INT PCR
  source 1..25: mol_type = other DNA
tgcaggggaacggggctcagtctga

SEQ ID NO: 20 - DNA, 20 bp, synthetic construct
  misc_feature 1..20: note = AAVS1 3'-BB PCR
  source 1..20: mol_type = other DNA
atgcttccggctcgtatgtt

SEQ ID NO: 21 - DNA, 22 bp, synthetic construct
  misc_feature 1..22: note = CNP Fw
  source 1..22: mol_type = other DNA
tcctcatcatgaacagaggctt

SEQ ID NO: 22 - DNA, 20 bp, synthetic construct
  misc_feature 1..20: note = CNP Rev
  source 1..20: mol_type = other DNA
aaactgcagctcaggcttgt

SEQ ID NO: 23 - DNA, 20 bp, synthetic construct
  misc_feature 1..20: note = DES Fw
  source 1..20: mol_type = other DNA
ccaacaagaacaacgacgcc

SEQ ID NO: 24 - DNA, 21 bp, synthetic construct
  misc_feature 1..21: note = DES Rev
  source 1..21: mol_type = other DNA
atcagggaatcgttagtgccc

SEQ ID NO: 25 - DNA, 22 bp, synthetic construct
  misc_feature 1..22: note = DMD Fw
  source 1..22: mol_type = other DNA
tggtgggaagaagtagaggact

SEQ ID NO: 26 - DNA, 20 bp, synthetic construct
  misc_feature 1..20: note = DMD Rev
  source 1..20: mol_type = other DNA
tgctgcttcccaaacttaga

SEQ ID NO: 27 - DNA, 20 bp, synthetic construct
  misc_feature 1..20: note = EGFP Fw
  source 1..20: mol_type = other DNA
cccgacaaccactacctgag

SEQ ID NO: 28 - DNA, 20 bp, synthetic construct
  misc_feature 1..20: note = EGFP Rev
  source 1..20: mol_type = other DNA
gtccatgccgagagtgatcc

SEQ ID NO: 29 - DNA, 20 bp, synthetic construct
  misc_feature 1..20: note = FOXG1 Fw
  source 1..20: mol_type = other DNA
tgccaagttttacgacggga

SEQ ID NO: 30 - DNA, 20 bp, synthetic construct
  misc_feature 1..20: note = FOXG1 Rev
  source 1..20: mol_type = other DNA
gggttggaagaagacccctg

SEQ ID NO: 31 - DNA, 20 bp, synthetic construct
  misc_feature 1..20: note = GRIA4 Fw
  source 1..20: mol_type = other DNA
ggccagggaattgacatgga

SEQ ID NO: 32 - DNA, 23 bp, synthetic construct
  misc_feature 1..23: note = GRIA4 Rev
  source 1..23: mol_type = other DNA
aaccaacctttctaggtcctgtg

SEQ ID NO: 33 - DNA, 20 bp, synthetic construct
  misc_feature 1..20: note = HMBS (PBGD) Fw
  source 1..20: mol_type = other DNA
attaccccgggagactgaac

SEQ ID NO: 34 - DNA, 20 bp, synthetic construct
  misc_feature 1..20: note = HMBS (PBGD) Rev
  source 1..20: mol_type = other DNA
ggctgttgcttggacttctc

SEQ ID NO: 35 - DNA, 20 bp, synthetic construct
  misc_feature 1..20: note = MAG Fw
  source 1..20: mol_type = other DNA
cagaagacgtccccaactca

SEQ ID NO: 36 - DNA, 22 bp, synthetic construct
  misc_feature 1..22: note = MAG Rev
  source 1..22: mol_type = other DNA
cctcgggaggctgaaatcataa

SEQ ID NO: 37 - DNA, 21 bp, synthetic construct
  misc_feature 1..21: note = MAP2 Fw
  source 1..21: mol_type = other DNA
agactgcagctctgcctttag

SEQ ID NO: 38 - DNA, 23 bp, synthetic construct
  misc_feature 1..23: note = MAP2 Rev
  source 1..23: mol_type = other DNA
aggctgtaagtaaatcttcctcc

SEQ ID NO: 39 - DNA, 24 bp, synthetic construct
  misc_feature 1..24: note = MBP Fw
  source 1..24: mol_type = other DNA
tggtgatggagatgtcaagcaggt

SEQ ID NO: 40 - DNA, 24 bp, synthetic construct
  misc_feature 1..24: note = MBP Rev
  source 1..24: mol_type = other DNA
gctgtggtttggaaacgaggttgt

SEQ ID NO: 41 - DNA, 23 bp, synthetic construct
  misc_feature 1..23: note = MOG Fw
  source 1..23: mol_type = other DNA
agagatagagaatctccaccgga

SEQ ID NO: 42 - DNA, 21 bp, synthetic construct
  misc_feature 1..21: note = MOG Rev
  source 1..21: mol_type = other DNA
tgatcaaggcaaccaagggtc

SEQ ID NO: 43 - DNA, 22 bp, synthetic construct
  misc_feature 1..22: note = MYH1 Fw
  source 1..22: mol_type = other DNA
cacactagtttcacagctctcg

SEQ ID NO: 44 - DNA, 20 bp, synthetic construct
  misc_feature 1..20: note = MYH1 Rev
  source 1..20: mol_type = other DNA
cagggcactcttggccttta

SEQ ID NO: 45 - DNA, 21 bp, synthetic construct
  misc_feature 1..21: note = MYH2 Fw
  source 1..21: mol_type = other DNA
ggaagctctggtgtctcagtt

SEQ ID NO: 46 - DNA, 21 bp, synthetic construct
  misc_feature 1..21: note = MYH2 Rev
  source 1..21: mol_type = other DNA
cagggcgttcttggcttttat

SEQ ID NO: 47 - DNA, 20 bp, synthetic construct
  misc_feature 1..20: note = MYH3 Fw
  source 1..20: mol_type = other DNA
gctgcatacccagaacacca

SEQ ID NO: 48 - DNA, 20 bp, synthetic construct
  misc_feature 1..20: note = MYH3 Rev
  source 1..20: mol_type = other DNA
ccctgctggcatcttctacc

SEQ ID NO: 49 - DNA, 20 bp, synthetic construct
  misc_feature 1..20: note = MYH4 Fw
  source 1..20: mol_type = other DNA
tcgcatttgtcagccaaggg

SEQ ID NO: 50 - DNA, 21 bp, synthetic construct
  misc_feature 1..21: note = MYH4 Rev
  source 1..21: mol_type = other DNA
tgaaacccaggatgtccacag

SEQ ID NO: 51 - DNA, 20 bp, synthetic construct
  misc_feature 1..20: note = MYH7 Fw
  source 1..20: mol_type = other DNA
gagactgtcgtgggcttgta

SEQ ID NO: 52 - DNA, 21 bp, synthetic construct
  misc_feature 1..21: note = MYH7 Rev
  source 1..21: mol_type = other DNA
gcccttctcaataggcgcatc

SEQ ID NO: 53 - DNA, 20 bp, synthetic construct
  misc_feature 1..20: note = MYH8 Fw
  source 1..20: mol_type = other DNA
tgaagcagatagcagcgcga

SEQ ID NO: 54 - DNA, 20 bp, synthetic construct
  misc_feature 1..20: note = MYH8 Rev
  source 1..20: mol_type = other DNA
cgtacgaagtgagggtgtgt

SEQ ID NO: 55 - DNA, 20 bp, synthetic construct
  misc_feature 1..20: note = MYOD1 (endo) Fw
  source 1..20: mol_type = other DNA
gccgctttccttaaccacaa

SEQ ID NO: 56 - DNA, 20 bp, synthetic construct
  misc_feature 1..20: note = MYOD1 (endo) Rev
  source 1..20: mol_type = other DNA
ctgaatgcccacccactgtc

SEQ ID NO: 57 - DNA, 20 bp, synthetic construct
  misc_feature 1..20: note = MYOD1 Fw
  source 1..20: mol_type = other DNA
cgacggcatgatggactaca

SEQ ID NO: 58 - DNA, 20 bp, synthetic construct
  misc_feature 1..20: note = MYOD1 Rev
  source 1..20: mol_type = other DNA
tagtaggcgccttcgtagca

SEQ ID NO: 59 - DNA, 22 bp, synthetic construct
  misc_feature 1..22: note = NANOG Fw
  source 1..22: mol_type = other DNA
agcagatgcaagaactctccaa

SEQ ID NO: 60 - DNA, 20 bp, synthetic construct
  misc_feature 1..20: note = NANOG Rev
  source 1..20: mol_type = other DNA
tgaggccttctgcgtcacac

SEQ ID NO: 61 - DNA, 21 bp, synthetic construct
  misc_feature 1..21: note = NEUROG2 (NGN2) Fw
  source 1..21: mol_type = other DNA
tgttcgtcaaatccgagacct

SEQ ID NO: 62 - DNA, 20 bp, synthetic construct
  misc_feature 1..20: note = NEUROG2 (NGN2) Rev
  source 1..20: mol_type = other DNA
cgatccgagcagcactaaca

SEQ ID NO: 63 - DNA, 20 bp, synthetic construct
  misc_feature 1..20: note = PAX6 Fw
  source 1..20: mol_type = other DNA
cgagatttcagagccccata

SEQ ID NO: 64 - DNA, 20 bp, synthetic construct
  misc_feature 1..20: note = PAX6 Rev
  source 1..20: mol_type = other DNA
aagacaccaccgagctgatt

SEQ ID NO: 65 - DNA, 22 bp, synthetic construct
  misc_feature 1..22: note = PLP Fw
  source 1..22: mol_type = other DNA
aacagctgagttccaaatgacc

SEQ ID NO: 66 - DNA, 20 bp, synthetic construct
  misc_feature 1..20: note = PLP Rev
  source 1..20: mol_type = other DNA
acggcaaagttgtaagtggc

SEQ ID NO: 67 - DNA, 20 bp, synthetic construct
  misc_feature 1..20: note = POU3F2 (BRN2) Fw
  source 1..20: mol_type = other DNA
acccgctttatcgaaggcaa

SEQ ID NO: 68 - DNA, 20 bp, synthetic construct
  misc_feature 1..20: note = POU3F2 (BRN2) Rev
  source 1..20: mol_type = other DNA
cctccataacctcccccaga

SEQ ID NO: 69 - DNA, 20 bp, synthetic construct
  misc_feature 1..20: note = POU5F1 (OCT4) Fw
  source 1..20: mol_type = other DNA
gtggaggaagctgacaacaa

SEQ ID NO: 70 - DNA, 20 bp, synthetic construct
  misc_feature 1..20: note = POU5F1 (OCT4) Rev
  source 1..20: mol_type = other DNA
attctccaggttgcctctca

SEQ ID NO: 71 - DNA, 20 bp, synthetic construct
  misc_feature 1..20: note = RYR1 Fw
  source 1..20: mol_type = other DNA
caatcgccagaacggagaga

SEQ ID NO: 72 - DNA, 20 bp, synthetic construct
  misc_feature 1..20: note = RYR1 Rev
  source 1..20: mol_type = other DNA
gtcgtgttccctgtctgtgt

SEQ ID NO: 73 - DNA, 20 bp, synthetic construct
  misc_feature 1..20: note = SLC17A6 (VGLUT2) Fw
  source 1..20: mol_type = other DNA
gtagactggcaaccacctcc

SEQ ID NO: 74 - DNA, 22 bp, synthetic construct
  misc_feature 1..22: note = SLC17A6 (VGLUT2) Rev
  source 1..22: mol_type = other DNA
ccattccaaagcttccgtagac

SEQ ID NO: 75 - DNA, 22 bp, synthetic construct
  misc_feature 1..22: note = SYP Fw
  source 1..22: mol_type = other DNA
acctcgggactcaacacctcgg

SEQ ID NO: 76 - DNA, 22 bp, synthetic construct
  misc_feature 1..22: note = SYP Rev
  source 1..22: mol_type = other DNA
gaaccacaggttgccgacccag

SEQ ID NO: 77 - DNA, 20 bp, synthetic construct
  misc_feature 1..20: note = SYN1 Fw
  source 1..20: mol_type = other DNA
ccctgggtgtttgcccagat

SEQ ID NO: 78 - DNA, 20 bp, synthetic construct
  misc_feature 1..20: note = SYN1 Rev
  source 1..20: mol_type = other DNA
accacggggtacgttgtact

SEQ ID NO: 79 - DNA, 21 bp, synthetic construct
  misc_feature 1..21: note = TUBB3 Fw
  source 1..21: mol_type = other DNA
caaccagatcggggccaagtt

SEQ ID NO: 80 - DNA, 19 bp, synthetic construct
  misc_feature 1..19: note = TUBB3 Rev
  source 1..19: mol_type = other DNA
ccgagtcgcccacgtagtt

SEQ ID NO: 81 - DNA, 52 bp, synthetic construct
  misc_feature 1..52: note = AAVS1 targeting vector Fw
  source 1..52: mol_type = other DNA
gtgatagagatccctggtgcaggtggactgactcacctgcacctgttttaga

SEQ ID NO: 82 - DNA, 52 bp, synthetic construct
  misc_feature 1..52: note = AAVSI targeting vector Rev
  source 1..52: mol_type = other DNA
actaaaacaggtgcaggtgagtcagtccacctgcaccagggatctctatcac

SEQ ID NO: 83-84 - skipped (2 entries)

SEQ ID NO: 85 - DNA, 268 bp, synthetic construct
  misc_feature 1..268: note = H1 POLIII Promoter H1-TO
  source 1..268: mol_type = other DNA
cgaacgctgacgtcatcaacccgctccaaggaatcgcgggcccagtgtcactaggcgggaacacccagcgcgcgtgcgccctggcaggaagatggctgtgagggacaggggagtggcgccctgcaatatttgcatgtcgctatgtgttctgggaaatcaccataaacgtgaaatgtctttggatttgggaatcttataagttccctatcagtgatagagatccctggtgcaggtggactgactcacctgcacctgttttagagctaga

SEQ ID NO: 86 - DNA, 268 bp, synthetic construct
  misc_feature 1..268: note = H1 POLIII Promoter H1-2TO
  source 1..268: mol_type = other DNA
cgaacgctgacgtcatcaacccgctccaaggaatcgcgggcccagtgtcactaggcgggaacacccagcgcgcgtgcgccctggcaggaagatggctgtgagggacaggggagtggcgccctgcaatatttgcatgtcgctatgtgttctgggaaatcaccataaacgtgaaatccctatcagtgatagagacttataagttccctatcagtgatagagatccctggtgcaggtggactgactcacctgcacctgttttagagctaga

SEQ ID NO: 87 - DNA, 23 bp, synthetic construct
  source 1..23: mol_type = other DNA
gtcgagtcgcttctcgattatgg

SEQ ID NO: 88 - DNA, 23 bp, synthetic construct
  source 1..23: mol_type = other DNA
ggcgatgacgagatcacgcgagg